European Patent Application EP 4 218 420 A1, published August 2, 2023. Title: Anti-coccidial composition comprising ginkgo leaf and uses thereof. Applicant: CJ CheilJedang Corporation. The sequence listing filed with the application follows.

SEQUENCE LISTING (2 sequences)

SEQ ID NO: 1 - DNA, 20 bp, Artificial Sequence
  synthetic_E. tenella ITS-1 forward primer
tggaggggattatgagagga

SEQ ID NO: 2 - DNA, 20 bp, Artificial Sequence
  synthetic_E. tenella ITS-1 reverse primer
caagcagcatgtaacggaga